European Patent Application EP 4 332 112 A1, published March 6, 2024. Title: peptide fragment and use thereof. Applicant: TOAGOSEI CO.,LTD. The sequence listing filed with the application follows.

SEQUENCE LISTING (6 sequences)

SEQ ID NO: 1 - protein, 7 aa, Artificial Sequence
  synthetic peptide
VVKSLVK

SEQ ID NO: 2 - protein, 13 aa, Artificial Sequence
  synthetic peptide
KKRTLRKNDRKKR

SEQ ID NO: 3 - protein, 15 aa, Artificial Sequence
  synthetic peptide
TLKERCLQVVRSLVK

SEQ ID NO: 4 - protein, 14 aa, Artificial Sequence
  synthetic peptide
VVKSLVKVVKSLVK

SEQ ID NO: 5 - protein, 14 aa, Artificial Sequence
  synthetic peptide
VVRSLVKVVRSLVK

SEQ ID NO: 6 - protein, 14 aa, Artificial Sequence
  synthetic peptide
VVRSLVRVVRSLVR